European Patent Specification EP 3 470 997 B1, published October 23, 2024. Title: METHOD FOR USING DNA TO STORE TEXT INFORMATION, DECODING METHOD THEREFOR AND APPLICATION THEREOF. Applicant: BGI SHENZHEN. The sequence listing filed with the application follows.

SEQUENCE LISTING (44 sequences)

SEQ ID NO: 1 - DNA, 25 bp, Artificial Sequence
atagcttaacgcgtatgacatcgca

SEQ ID NO: 2 - DNA, 25 bp, Artificial Sequence
gtgcgatgtcatacgcgttaagcta

SEQ ID NO: 3 - DNA, 25 bp, Artificial Sequence
atacaagcttcagacagttgtggtg

SEQ ID NO: 4 - DNA, 25 bp, Artificial Sequence
gcaccacaactgtctgaagcttgta

SEQ ID NO: 5 - DNA, 25 bp, Artificial Sequence
aatgtcatggttgtgacgtgcatac

SEQ ID NO: 6 - DNA, 25 bp, Artificial Sequence
ggtatgcacgtcacaaccatgacat

SEQ ID NO: 7 - DNA, 25 bp, Artificial Sequence
atagcttgagaccattacgtacggt

SEQ ID NO: 8 - DNA, 25 bp, Artificial Sequence
gaccgtacgtaatggtctcaagcta

SEQ ID NO: 9 - DNA, 25 bp, Artificial Sequence
atagctaaccaacaccactagagct

SEQ ID NO: 10 - DNA, 25 bp, Artificial Sequence
gagctctagtggtgttggttagcta

SEQ ID NO: 11 - DNA, 25 bp, Artificial Sequence
atagctaatccggaacttgtggtgt

SEQ ID NO: 12 - DNA, 25 bp, Artificial Sequence
gacaccacaagttccggattagcta

SEQ ID NO: 13 - DNA, 25 bp, Artificial Sequence
atacgattggatcctagtacggtag

SEQ ID NO: 14 - DNA, 25 bp, Artificial Sequence
gctaccgtactaggatccaatcgta

SEQ ID NO: 15 - DNA, 8 bp, Artificial Sequence
ctcattcc

SEQ ID NO: 16 - DNA, 9 bp, Artificial Sequence
tggaatgag

SEQ ID NO: 17 - DNA, 8 bp, Artificial Sequence
aattcgcg

SEQ ID NO: 18 - DNA, 9 bp, Artificial Sequence
tcgcgaatt

SEQ ID NO: 19 - DNA, 9 bp, Artificial Sequence
caattcgcg

SEQ ID NO: 20 - DNA, 8 bp, Artificial Sequence
cgcgaatt

SEQ ID NO: 21 - DNA, 8 bp, Artificial Sequence
cctttagc

SEQ ID NO: 22 - DNA, 9 bp, Artificial Sequence
tgctaaagg

SEQ ID NO: 23 - DNA, 9 bp, Artificial Sequence
ccctttagc

SEQ ID NO: 24 - DNA, 8 bp, Artificial Sequence
gctaaagg

SEQ ID NO: 25 - DNA, 8 bp, Artificial Sequence
acagagac

SEQ ID NO: 26 - DNA, 9 bp, Artificial Sequence
tgtctctgt

SEQ ID NO: 27 - DNA, 9 bp, Artificial Sequence
cacagagac

SEQ ID NO: 28 - DNA, 8 bp, Artificial Sequence
gtctctgt

SEQ ID NO: 29 - DNA, 8 bp, Artificial Sequence
ccgtcata

SEQ ID NO: 30 - DNA, 9 bp, Artificial Sequence
ttatgacgg

SEQ ID NO: 31 - DNA, 9 bp, Artificial Sequence
cccgtcata

SEQ ID NO: 32 - DNA, 8 bp, Artificial Sequence
tatgacgg

SEQ ID NO: 33 - DNA, 8 bp, Artificial Sequence
ggatctac

SEQ ID NO: 34 - DNA, 9 bp, Artificial Sequence
tgtagatcc

SEQ ID NO: 35 - DNA, 9 bp, Artificial Sequence
cggatctac

SEQ ID NO: 36 - DNA, 8 bp, Artificial Sequence
gtagatcc

SEQ ID NO: 37 - DNA, 8 bp, Artificial Sequence
gttgcatc

SEQ ID NO: 38 - DNA, 9 bp, Artificial Sequence
tgatgcaac

SEQ ID NO: 39 - DNA, 9 bp, Artificial Sequence
cgttgcatc

SEQ ID NO: 40 - DNA, 8 bp, Artificial Sequence
gatgcaac

SEQ ID NO: 41 - DNA, 9 bp, Artificial Sequence
catcgggaa

SEQ ID NO: 42 - DNA, 8 bp, Artificial Sequence
ttcccgat

SEQ ID NO: 43 - DNA, 59 bp, Artificial Sequence
gcgcgcttggttcagacgtgagaagtgatgcacagtagcttaacgcgtatgacatcgca

SEQ ID NO: 44 - DNA, 27 bp, Artificial Sequence
gcgcgctaccgtactaggatccaatcg